European Patent Application EP 4 442 283 A1, published October 9, 2024. Title: ANTI-HUMAN TROP2 ANTIBODY-CAMPTOTHECIN DRUG CONJUGATE AND MEDICAL USE THEREOF. Applicant: BAILI-BIO (CHENGDU) PHARMACEUTICAL CO., LTD. Application WO PCT/CN2022/136278, filed December 2, 2022. The sequence listing filed with the application follows.

SEQUENCE LISTING (44 sequences)

SEQ ID NO: 1 - protein, 8 aa, synthetic construct
GYTFTSFD

SEQ ID NO: 2 - protein, 7 aa, synthetic construct
IFPGDGN

SEQ ID NO: 3 - protein, 11 aa, synthetic construct
VRGEALYYFDY

SEQ ID NO: 4 - protein, 8 aa, synthetic construct
GYTFTDHV

SEQ ID NO: 5 - protein, 8 aa, synthetic construct
IYPGSDNS

SEQ ID NO: 6 - protein, 18 aa, synthetic construct
AREGYGYGKNGVGYAMDY

SEQ ID NO: 7 - protein, 6 aa, synthetic construct
QDINKY

SEQ ID NO: 8 - skipped

SEQ ID NO: 9 - protein, 8 aa, synthetic construct
LQYDDLFT

SEQ ID NO: 10 - protein, 6 aa, synthetic construct
QSVSND

SEQ ID NO: 11 - skipped

SEQ ID NO: 12 - protein, 9 aa, synthetic construct
QQDYSSPWT

SEQ ID NO: 13 - protein, 118 aa, synthetic construct
QVQLVQSGAEVKKPGASVKLSCKASGYTFTSFDINWVRQAPEQRLEWMGWIFPGDGNTKYSQKFQGRATITRDTSASTAYMELSSLRSEDTAVYYCVRGEALYYFDYWGQGTLVTVSS

SEQ ID NO: 14 - protein, 106 aa, synthetic construct
DIQMTQSPSSLSASVGDRVTITCRASQDINKYLAWYQQKPGKVPKLLIYSTSTLQSGVPSRFSGSGSGTDFTLTISSLQPEDVATYYCLQYDDLFTFGQGTKLEIK

SEQ ID NO: 15 - protein, 125 aa, synthetic construct
QVQLVQSGAEVKKPGASVKVSCKASGYTFTDHVISWVRQATGQGLEWMGQIYPGSDNSYYAQKFQGRVTLTADKSINTAYMELSSLRSEDTAVYYCAREGYGYGKNGVGYAMDYWGQGTLVTVSS

SEQ ID NO: 16 - protein, 107 aa, synthetic construct
DIVMTQSPDSLAVSLGERATINCKASQSVSNDVVWYQQKPGQPPKLLIYYASNRYTGVPDRFSGSGYGTDFTLTISSLQAEDVAVYYCQQDYSSPWTFGGGTKVEIK

SEQ ID NO: 17 - protein, 447 aa, synthetic construct
QVQLVQSGAEVKKPGASVKLSCKASGYTFTSFDINWVRQAPEQRLEWMGWIFPGDGNTKYSQKFQGRATITRDTSASTAYMELSSLRSEDTAVYYCVRGEALYYFDYWGQGTLVTVSSASTKGPSVFPLAPSSKSTSGGTAALGCLVKDYFPEPVTVSWNSGALTSGVHTFPAVLQSSGLYSLSSVVTVPSSSLGTQTYICNVNHKPSNTKVDKRVEPKSCDKTHTCPPCPAPELLGGPSVFLFPPKPKDTLMISRTPEVTCVVVDVSHEDPEVKFNWYVDGVEVHNAKTKPREEQYNSTYRVVSVLTVLHQDWLNGKEYKCKVSNKALPAPIEKTISKAKGQPREPQVYTLPPSRDELTKNQVSLTCLVKGFYPSDIAVEWESNGQPENNYKTTPPVLDSDGSFFLYSKLTVDKSRWQQGNVFSCSVMHEALHNHYTQKSLSLSPG

SEQ ID NO: 18 - protein, 213 aa, synthetic construct
DIQMTQSPSSLSASVGDRVTITCRASQDINKYLAWYQQKPGKVPKLLIYSTSTLQSGVPSRFSGSGSGTDFTLTISSLQPEDVATYYCLQYDDLFTFGQGTKLEIKRTVAAPSVFIFPPSDEQLKSGTASVVCLLNNFYPREAKVQWKVDNALQSGNSQESVTEQDSKDSTYSLSSTLTLSKADYEKHKVYACEVTHQGLSSPVTKSFNRGEC

SEQ ID NO: 19 - protein, 454 aa, synthetic construct
QVQLVQSGAEVKKPGASVKVSCKASGYTFTDHVISWVRQATGQGLEWMGQIYPGSDNSYYAQKFQGRVTLTADKSINTAYMELSSLRSEDTAVYYCAREGYGYGKNGVGYAMDYWGQGTLVTVSSASTKGPSVFPLAPSSKSTSGGTAALGCLVKDYFPEPVTVSWNSGALTSGVHTFPAVLQSSGLYSLSSVVTVPSSSLGTQTYICNVNHKPSNTKVDKRVEPKSCDKTHTCPPCPAPELLGGPSVFLFPPKPKDTLMISRTPEVTCVVVDVSHEDPEVKFNWYVDGVEVHNAKTKPREEQYNSTYRVVSVLTVLHQDWLNGKEYKCKVSNKALPAPIEKTISKAKGQPREPQVYTLPPSRDELTKNQVSLTCLVKGFYPSDIAVEWESNGQPENNYKTTPPVLDSDGSFFLYSKLTVDKSRWQQGNVFSCSVMHEALHNHYTQKSLSLSPG

SEQ ID NO: 20 - protein, 214 aa, synthetic construct
DIVMTQSPDSLAVSLGERATINCKASQSVSNDVVWYQQKPGQPPKLLIYYASNRYTGVPDRFSGSGYGTDFTLTISSLQAEDVAVYYCQQDYSSPWTFGGGTKVEIKRTVAAPSVFIFPPSDEQLKSGTASVVCLLNNFYPREAKVQWKVDNALQSGNSQESVTEQDSKDSTYSLSSTLTLSKADYEKHKVYACEVTHQGLSSPVTKSFNRGEC

SEQ ID NO: 21 - DNA, 24 bp, synthetic construct
  source 1..24: mol_type = other DNA
ggctacaccttcacaagctttgat

SEQ ID NO: 22 - DNA, 21 bp, synthetic construct
  source 1..21: mol_type = other DNA
atttttcctggagatggtaat

SEQ ID NO: 23 - DNA, 33 bp, synthetic construct
  source 1..33: mol_type = other DNA
gtaagaggggaggccctgtattactttgactac

SEQ ID NO: 24 - DNA, 24 bp, synthetic construct
  source 1..24: mol_type = other DNA
ggatacacattcactgaccatgtc

SEQ ID NO: 25 - DNA, 24 bp, synthetic construct
  source 1..24: mol_type = other DNA
atttatcctggaagtgataatagt

SEQ ID NO: 26 - DNA, 54 bp, synthetic construct
  source 1..54: mol_type = other DNA
gcaagagagggctatggttatggaaaaaacggagttggctatgctatggactac

SEQ ID NO: 27 - DNA, 18 bp, synthetic construct
  source 1..18: mol_type = other DNA
caagacattaataagtat

SEQ ID NO: 28 - skipped

SEQ ID NO: 29 - DNA, 24 bp, synthetic construct
  source 1..24: mol_type = other DNA
ctgcagtatgatgatctattcacg

SEQ ID NO: 30 - DNA, 18 bp, synthetic construct
  source 1..18: mol_type = other DNA
cagagtgtgagtaatgat

SEQ ID NO: 31 - skipped

SEQ ID NO: 32 - DNA, 27 bp, synthetic construct
  source 1..27: mol_type = other DNA
cagcaggattattcctctccgtggacg

SEQ ID NO: 33 - DNA, 355 bp, synthetic construct
  source 1..355: mol_type = other DNA
caggtgcagctggtgcagtccggcgccgaggtgaagaagcccggcgcctccgtgaagctgagctgtaaggcctccggctacaccttcacctccttcgacattaactgggtgcggcaggcccccgagcagcgcctggagtggatgggctggatcttccccggcgacggcaacaccaagtactcccagaagttccagggaagagctaccatcaccagagatacatccgcttctacagcttacatggagctgtctagcctgagatctgaggatacagctgtgtattactgtgtgagaggagaggctctgtactattttgattattggggccagggcaccctggtgacagtgtcttctg

SEQ ID NO: 34 - DNA, 319 bp, synthetic construct
  source 1..319: mol_type = other DNA
gatatccagatgacccagtctccatctagcctgtccgcttctgtgggcgatagagtgaccatcacatgcagagcttctcaggatatcaataagtatctggcttggtatcagcagaagcctggaaaggtgcctaagctgctgatctactctacatctaccctgcagtctggagtgccttctagattttctggatctggctctggcaccgattttacactgacaatctcttctctgcagcctgaggatgtggctacatattattgtctgcagtatgatgatctgttcacctttggccagggcaccaagctggagatcaagc

SEQ ID NO: 35 - DNA, 376 bp, synthetic construct
  source 1..376: mol_type = other DNA
caggtgcagctggtgcagtctggggccgaggtgaaaaagccaggcgcttctgtgaaggtgtcttgcaaggcctccggctacaccttcaccgaccacgtgatctcctgggtgcgccaggccaccggccagggcctggagtggatgggccagatctaccccggctccgacaactcctactacgcccagaagttccagggcagggtgactctgaccgccgacaagtccatcaacaccgcctacatggagctgtcctccctgaggtccgaggacaccgccgtgtactactgcgccagggagggctacggctacggcaagaacggcgtgggctacgccatggattattggggccagggcaccctggtgacagtgtcttctg

SEQ ID NO: 36 - DNA, 322 bp, synthetic construct
  source 1..322: mol_type = other DNA
gatatcgtgatgacacagtctcctgattctctggccgtgtctctgggcgaaagagctacaatcaactgtaaggcttctcagtctgtgtctaatgatgtggtgtggtaccagcagaagcctgggcagccccccaagctgctgatctactacgcctccaacaggtacaccggcgtgcccgacaggttctccggctccggctacggcaccgacttcaccctgaccatctcctccctgcaggccgaggacgtggccgtgtactactgccagcaggactactcctccccctggaccttcggcggcggcaccaaggtggagatcaagc

SEQ ID NO: 37 - DNA, 1401 bp, synthetic construct
  source 1..1401: mol_type = other DNA
atgggctggtcctgggtgttcctgttcctgctgagcgtgaccgccggcgtgcactcccaggtgcagctggtgcagtccggcgccgaggtgaagaagcccggcgcctccgtgaagctgagctgtaaggcctccggctacaccttcacctccttcgacattaactgggtgcggcaggcccccgagcagcgcctggagtggatgggctggatcttccccggcgacggcaacaccaagtactcccagaagttccagggaagagctaccatcaccagagatacatccgcttctacagcttacatggagctgtctagcctgagatctgaggatacagctgtgtattactgtgtgagaggagaggctctgtactattttgattattggggccagggcaccctggtgacagtgtcttctgctagcaccaagggcccatcggtcttccccctggcaccctcctccaagagcacctctgggggcacagcggccctgggctgcctggtcaaggactacttccccgaaccggtgacggtgtcgtggaactcaggcgccctgaccagcggcgtgcacaccttcccggctgtcctacagtcctcaggactctactccctcagcagcgtggtgaccgtgccctccagcagcttgggcacccagacctacatctgcaacgtgaatcacaagcccagcaacaccaaggtggacaagagagttgagcccaaatcttgtgacaaaactcacacatgcccaccgtgcccagcacctgaactcctggggggaccgtcagtcttcctcttccccccaaaacccaaggacaccctcatgatctcccggacccctgaggtcacatgcgtggtggtggacgtgagccacgaagaccctgaggtcaagttcaactggtacgtggacggcgtggaggtgcataatgccaagacaaagccgcgggaggagcagtacaacagcacgtaccgtgtggtcagcgtcctcaccgtcctgcaccaggactggctgaatggcaaggagtacaagtgcaaggtctccaacaaagccctcccagcccccatcgagaaaaccatctccaaagccaaagggcagccccgagaaccacaggtgtacaccctgcccccatcccgggatgagctgaccaagaaccaggtcagcctgacctgcctggtcaaaggcttctatcccagcgacatcgccgtggagtgggagagcaatgggcagccggagaacaactacaagaccacgcctcccgtgctggactccgacggctccttcttcctctatagcaagctcaccgtggacaagagcaggtggcagcaggggaacgtcttctcatgctccgtgatgcatgaggctctgcacaaccactacacgcagaagagcctctccctgtctccgggttaa

SEQ ID NO: 38 - DNA, 642 bp, synthetic construct
  source 1..642: mol_type = other DNA
gatatccagatgacccagtctccatctagcctgtccgcttctgtgggcgatagagtgaccatcacatgcagagcttctcaggatatcaataagtatctggcttggtatcagcagaagcctggaaaggtgcctaagctgctgatctactctacatctaccctgcagtctggagtgccttctagattttctggatctggctctggcaccgattttacactgacaatctcttctctgcagcctgaggatgtggctacatattattgtctgcagtatgatgatctgttcacctttggccagggcaccaagctggagatcaagcgtacggtggctgcaccatctgtcttcatcttcccgccatctgatgagcagttgaaatctggaactgcctctgttgtgtgcctgctgaataacttctatcccagagaggccaaagtacagtggaaggtggataacgccctccaatcgggtaactcccaggagagtgtcacagagcaggacagcaaggacagcacctacagcctcagcagcaccctgacgctgagcaaagcagactacgagaaacacaaagtctacgcctgcgaagtcacccatcagggcctgagctcgcccgtcacaaagagcttcaacaggggagagtgttag

SEQ ID NO: 39 - DNA, 1365 bp, synthetic construct
  source 1..1365: mol_type = other DNA
caggtgcagctggtgcagtctggggccgaggtgaaaaagccaggcgcttctgtgaaggtgtcttgcaaggcctccggctacaccttcaccgaccacgtgatctcctgggtgcgccaggccaccggccagggcctggagtggatgggccagatctaccccggctccgacaactcctactacgcccagaagttccagggcagggtgactctgaccgccgacaagtccatcaacaccgcctacatggagctgtcctccctgaggtccgaggacaccgccgtgtactactgcgccagggagggctacggctacggcaagaacggcgtgggctacgccatggattattggggccagggcaccctggtgacagtgtcttctgctagcaccaagggcccatcggtcttccccctggcaccctcctccaagagcacctctgggggcacagcggccctgggctgcctggtcaaggactacttccccgaaccggtgacggtgtcgtggaactcaggcgccctgaccagcggcgtgcacaccttcccggctgtcctacagtcctcaggactctactccctcagcagcgtggtgaccgtgccctccagcagcttgggcacccagacctacatctgcaacgtgaatcacaagcccagcaacaccaaggtggacaagagagttgagcccaaatcttgtgacaaaactcacacatgcccaccgtgcccagcacctgaactcctggggggaccgtcagtcttcctcttccccccaaaacccaaggacaccctcatgatctcccggacccctgaggtcacatgcgtggtggtggacgtgagccacgaagaccctgaggtcaagttcaactggtacgtggacggcgtggaggtgcataatgccaagacaaagccgcgggaggagcagtacaacagcacgtaccgtgtggtcagcgtcctcaccgtcctgcaccaggactggctgaatggcaaggagtacaagtgcaaggtctccaacaaagccctcccagcccccatcgagaaaaccatctccaaagccaaagggcagccccgagaaccacaggtgtacaccctgcccccatcccgggatgagctgaccaagaaccaggtcagcctgacctgcctggtcaaaggcttctatcccagcgacatcgccgtggagtgggagagcaatgggcagccggagaacaactacaagaccacgcctcccgtgctggactccgacggctccttcttcctctatagcaagctcaccgtggacaagagcaggtggcagcaggggaacgtcttctcatgctccgtgatgcatgaggctctgcacaaccactacacgcagaagagcctctccctgtctccgggttaa

SEQ ID NO: 40 - DNA, 645 bp, synthetic construct
  source 1..645: mol_type = other DNA
gatatcgtgatgacacagtctcctgattctctggccgtgtctctgggcgaaagagctacaatcaactgtaaggcttctcagtctgtgtctaatgatgtggtgtggtaccagcagaagcctgggcagccccccaagctgctgatctactacgcctccaacaggtacaccggcgtgcccgacaggttctccggctccggctacggcaccgacttcaccctgaccatctcctccctgcaggccgaggacgtggccgtgtactactgccagcaggactactcctccccctggaccttcggcggcggcaccaaggtggagatcaagcgtacggtggctgcaccatctgtcttcatcttcccgccatctgatgagcagttgaaatctggaactgcctctgttgtgtgcctgctgaataacttctatcccagagaggccaaagtacagtggaaggtggataacgccctccaatcgggtaactcccaggagagtgtcacagagcaggacagcaaggacagcacctacagcctcagcagcaccctgacgctgagcaaagcagactacgagaaacacaaagtctacgcctgcgaagtcacccatcagggcctgagctcgcccgtcacaaagagcttcaacaggggagagtgttag

SEQ ID NO: 41 - DNA, 1410 bp, synthetic construct
  source 1..1410: mol_type = other DNA
atgaaacacctgtggttcttcctcctgctggtggcagctcccagatgggtgctgagccaggtgcagctggtgcagtctggcgccgaagtgaagaaaccaggcgccagcgtgaaggtgtcctgcaaggccagcggctacacctttaccaccgccggcatgcagtgggtgcgccaggctcctggacagggcctggaatggatgggctggatcaacacccacagcggcgtgcccaaatacgccgaggacttcaagggcagagtgaccatcagcgccgacaccagcacctccacagcctacctgcagctgagcagcctgaagtccgaggacaccgccgtgtactactgcgccagaagcggcttcggcagcagctactggtacttcgacgtgtggggccagggcaccctcgtgaccgtcagctcagcctccaccaagggcccaagcgtcttccccctggcaccctcctccaagagcacctctggcggcacagccgccctgggctgcctggtcaaggactacttccccgaacccgtgaccgtgagctggaactcaggcgccctgaccagcggcgtgcacaccttccccgctgtcctgcagtcctcaggactctactccctcagcagcgtggtgaccgtgccctccagcagcttgggcacccagacctacatctgcaacgtgaatcacaagcccagcaacaccaaggtggacaagagagttgagcccaaatcttgtgacaaaactcacacatgcccaccctgcccagcacctgaactcctggggggaccctcagtcttcctcttccccccaaaacccaaggacaccctcatgatctcccggacccctgaggtcacatgcgtggtggtggacgtgagccacgaagaccctgaggtcaagttcaactggtacgtggacggcgtggaggtgcataatgccaagacaaagccccgggaggagcagtacaacagcacgtaccgggtggtcagcgtcctcaccgtcctgcaccaggactggctgaatggcaaggagtacaagtgcaaggtctccaacaaagccctcccagcccccatcgagaaaaccatctccaaagccaaaggccagccccgggaaccacaggtgtacaccctgcccccatcccgggaggagatgaccaagaaccaggtcagcctgacctgcctggtcaaaggcttctatcccagcgacatcgccgtggagtgggagagcaatggccagcccgagaacaactacaagaccacccctcccgtgctggactccgacggctccttcttcctctacagcaagctcaccgtggacaagagcaggtggcagcagggcaacgtcttctcatgctccgtgatgcatgaggctctgcacaaccactacacccagaagagcctctccctgtctcccggcaaa

SEQ ID NO: 42 - protein, 470 aa, synthetic construct
MKHLWFFLLLVAAPRWVLSQVQLVQSGAEVKKPGASVKVSCKASGYTFTTAGMQWVRQAPGQGLEWMGWINTHSGVPKYAEDFKGRVTISADTSTSTAYLQLSSLKSEDTAVYYCARSGFGSSYWYFDVWGQGTLVTVSSASTKGPSVFPLAPSSKSTSGGTAALGCLVKDYFPEPVTVSWNSGALTSGVHTFPAVLQSSGLYSLSSVVTVPSSSLGTQTYICNVNHKPSNTKVDKRVEPKSCDKTHTCPPCPAPELLGGPSVFLFPPKPKDTLMISRTPEVTCVVVDVSHEDPEVKFNWYVDGVEVHNAKTKPREEQYNSTYRVVSVLTVLHQDWLNGKEYKCKVSNKALPAPIEKTISKAKGQPREPQVYTLPPSREEMTKNQVSLTCLVKGFYPSDIAVEWESNGQPENNYKTTPPVLDSDGSFFLYSKLTVDKSRWQQGNVFSCSVMHEALHNHYTQKSLSLSPGK

SEQ ID NO: 43 - DNA, 702 bp, synthetic construct
  source 1..702: mol_type = other DNA
atggtgctgcagacccaggtgttcatctccctgctgctgtggatctccggcgcgtacggcgacatccagatgacccagagccctagcagcctgagcgccagcgtgggcgacagagtgaccatcacatgcaaggccagccaggacgtgtccacagccgtggcctggtatcagcagaagcctggcaaggcccccaagctgctgatctacagcgccagctaccggtacaccggcgtgcccagcagattttctggcagcggctccggcaccgacttcaccctgacaatcagcagcctgcagcccgaggacttcgccgtgtactactgccagcagcactacatcacccccctgacctttggccagggcaccaagctggaaatcaagcgtacggtggccgccccctccgtgttcatcttccccccctccgacgagcagctgaagtccggcaccgcctccgtggtgtgcctgctgaataacttctaccccagagaggccaaggtgcagtggaaggtggacaacgccctgcagtccgggaactcccaggagagcgtgaccgagcaggacagcaaggacagcacctacagcctgagcagcaccctgaccctgagcaaagccgactacgagaagcacaaggtgtacgcctgcgaggtgacccaccagggcctgagctcccccgtcaccaagagcttcaacaggggggagtgt

SEQ ID NO: 44 - protein, 234 aa, synthetic construct
MVLQTQVFISLLLWISGAYGDIQMTQSPSSLSASVGDRVTITCKASQDVSTAVAWYQQKPGKAPKLLIYSASYRYTGVPSRFSGSGSGTDFTLTISSLQPEDFAVYYCQQHYITPLTFGQGTKLEIKRTVAAPSVFIFPPSDEQLKSGTASVVCLLNNFYPREAKVQWKVDNALQSGNSQESVTEQDSKDSTYSLSSTLTLSKADYEKHKVYACEVTHQGLSSPVTKSFNRGEC